European Patent Specification EP 3 896 451 B1, published June 26, 2024. Title: IDENTIFICATION OF THERAPEUTIC TARGETS FOR FACIOSCAPULOHUMERAL MUSCULAR DYSTROPHY. Applicant: University of Massachusetts. Application Divisional application of EP17867141.8. The sequence listing filed with the application follows.

SEQUENCE LISTING (55 sequences)

SEQ ID NO: 1 - DNA, 57 bp, Artificial Sequence
  Synthetic Polynucleotide
ccgggcctctgacatgcgatttgaactcgagttcaaatcgcatgtcagaggcttttt

SEQ ID NO: 2 - DNA, 57 bp, Artificial Sequence
  Synthetic Polynucleotide
ccgggcagagagtaatggtgtgttactcgagtaacacaccattactctctgcttttt

SEQ ID NO: 3 - DNA, 57 bp, Artificial Sequence
  Synthetic Polynucleotide
ccgggcccaagtcttggtatgctatctcgagatagcataccaagacttgggcttttt

SEQ ID NO: 4 - DNA, 57 bp, Artificial Sequence
  Synthetic Polynucleotide
ccggcgacataaacttgacatctttctcgagaaagatgtcaagtttatgtcgttttt

SEQ ID NO: 5 - DNA, 57 bp, Artificial Sequence
  Synthetic Polynucleotide
ccggcctgccaaataccataagaaactcgagtttcttatggtatttggcaggttttt

SEQ ID NO: 6 - DNA, 57 bp, Artificial Sequence
  Synthetic Polynucleotide
ccggcgtactttgtttatcccagaactcgagttctgggataaacaaagtacgttttt

SEQ ID NO: 7 - DNA, 57 bp, Artificial Sequence
  Synthetic Polynucleotide
ccgggttctttaatttacgggtcttctcgagaagacccgtaaattaaagaacttttt

SEQ ID NO: 8 - DNA, 57 bp, Artificial Sequence
  Synthetic Polynucleotide
ccggccgggcaaatagattcgagtactcgagtactcgaatctatttgcccggttttt

SEQ ID NO: 9 - DNA, 58 bp, Artificial Sequence
  Synthetic Polynucleotide
ccgggcgatgaagaagaaggtcaaactcgagtttgaccttcttcttcatcgctttttg

SEQ ID NO: 10 - DNA, 57 bp, Artificial Sequence
  Synthetic Polynucleotide
ccggccctttgctgtgacacttcttctcgagaagaagtgtcacagcaaagggttttt

SEQ ID NO: 11 - DNA, 57 bp, Artificial Sequence
  Synthetic Polynucleotide
ccgggccctctttacgtgattcaaactcgagtttgaatcacgtaaagagggcttttt

SEQ ID NO: 12 - DNA, 25 bp, Artificial Sequence
  Synthetic Polynucleotide
cgttaccggggtggagcctcggaat

SEQ ID NO: 13 - DNA, 25 bp, Artificial Sequence
  Synthetic Polynucleotide
cttgcccggaagcgctggctggggt

SEQ ID NO: 14 - DNA, 25 bp, Artificial Sequence
  Synthetic Polynucleotide
gccaaagcagggaaacgggaggggt

SEQ ID NO: 15 - DNA, 25 bp, Artificial Sequence
  Synthetic Polynucleotide
atacaagttaaatcgtaattggaat

SEQ ID NO: 16 - DNA, 25 bp, Artificial Sequence
  Synthetic Polynucleotide
ttgactacacgatgggaaaagggat

SEQ ID NO: 17 - DNA, 25 bp, Artificial Sequence
  Synthetic Polynucleotide
aaaaccgtgagacttcacttggggt

SEQ ID NO: 18 - DNA, 25 bp, Artificial Sequence
  Synthetic Polynucleotide
tgtgtcttctgtgcctgacaggggt

SEQ ID NO: 19 - DNA, 23 bp, Artificial Sequence
  Synthetic Polynucleotide
gccctcacgcgtaccttcaacgg

SEQ ID NO: 20 - protein, 1082 aa, Artificial Sequence
  Synthetic Polypeptide
MAPKKKRKVGIHGVPAAKRNYILGLDIGITSVGYGIIDYETRDVIDAGVRLFKEANVENNEGRRSKRGARRLKRRRRHRIQRVKKLLFDYNLLTDHSELSGINPYEARVKGLSQKLSEEEFSAALLHLAKRRGVHNVNEVEEDTGNELSTKEQISRNSKALEEKYVAELQLERLKKDGEVRGSINRFKTSDYVKEAKQLLKVQKAYHQLDQSFIDTYIDLLETRRTYYEGPGEGSPFGWKDIKEWYEMLMGHCTYFPEELRSVKYAYNADLYNALNDLNNLVITRDENEKLEYYEKFQIIENVFKQKKKPTLKQIAKEILVNEEDIKGYRVTSTGKPEFTNLKVYHDIKDITARKEIIENAELLDQIAKILTIYQSSEDIQEELTNLNSELTQEEIEQISNLKGYTGTHNLSLKAINLILDELWHTNDNQIAIFNRLKLVPKKVDLSQQKEIPTTLVDDFILSPVVKRSFIQSIKVINAIIKKYGLPNDIIIELAREKNSKDAQKMINEMQKRNRQTNERIEEIIRTTGKENAKYLIEKIKLHDMQEGKCLYSLEAIPLEDLLNNPFNYEVDHIIPRSVSFDNSFNNKVLVKQEENSKKGNRTPFQYLSSSDSKISYETFKKHILNLAKGKGRISKTKKEYLLEERDINRFSVQKDFINRNLVDTRYATRGLMNLLRSYFRVNNLDVKVKSINGGFTSFLRRKWKFKKERNKGYKHHAEDALIIANADFIFKEWKKLDKAKKVMENQMFEEKQAESMPEIETEQEYKEIFITPHQIKHIKDFKDYKYSHRVDKKPNRELINDTLYSTRKDDKGNTLIVNNLNGLYDKDNDKLKKLINKSPEKLLMYHHDPQTYQKLKLIMEQYGDEKNPLYKYYEETGNYLTKYSKKDNGPVIKKIKYYGNKLNAHLDITDDYPNSRNKVVKLSLKPYRFDVYLDNGVYKFVTVKNLDVIKKENYYEVNSKCYEEAKKLKKISNQAEFIASFYNNDLIKINGELYRVIGVNNDLLNRIEVNMIDITYREYLENMNDKRPPRIIKTIASKTQSIKKYSTDILGNLYEVKSKKHPQIIKKGKRPAATKKAGQAK

SEQ ID NO: 21 - protein, 1158 aa, Artificial Sequence
  Synthetic Polypeptide
MAPKKKRKVGIHGVPAAKRNYILGLAIGITSVGYGIIDYETRDVIDAGVRLFKEANVENNEGRRSKRGARRLKRRRRHRIQRVKKLLFDYNLLTDHSELSGINPYEARVKGLSQKLSEEEFSAALLHLAKRRGVHNVNEVEEDTGNELSTKEQISRNSKALEEKYVAELQLERLKKDGEVRGSINRFKTSDYVKEAKQLLKVQKAYHQLDQSFIDTYIDLLETRRTYYEGPGEGSPFGWKDIKEWYEMLMGHCTYFPEELRSVKYAYNADLYNALNDLNNLVITRDENEKLEYYEKFQIIENVFKQKKKPTLKQIAKEILVNEEDIKGYRVTSTGKPEFTNLKVYHDIKDITARKEIIENAELLDQIAKILTIYQSSEDIQEELTNLNSELTQEEIEQISNLKGYTGTHNLSLKAINLILDELWHTNDNQIAIFNRLKLVPKKVDLSQQKEIPTTLVDDFILSPVVKRSFIQSIKVINAIIKKYGLPNDIIIELAREKNSKDAQKMINEMQKRNRQTNERIEEIIRTTGKENAKYLIEKIKLHDMQEGKCLYSLEAIPLEDLLNNPFNYEVDHIIPRSVSFDNSFNNKVLVKQEEASKKGNRTPFQYLSSSDSKISYETFKKHILNLAKGKGRISKTKKEYLLEERDINRFSVQKDFINRNLVDTRYATRGLMNLLRSYFRVNNLDVKVKSINGGFTSFLRRKWKFKKERNKGYKHHAEDALIIANADFIFKEWKKLDKAKKVMENQMFEEKQAESMPEIETEQEYKEIFITPHQIKHIKDFKDYKYSHRVDKKPNRELINDTLYSTRKDDKGNTLIVNNLNGLYDKDNDKLKKLINKSPEKLLMYHHDPQTYQKLKLIMEQYGDEKNPLYKYYEETGNYLTKYSKKDNGPVIKKIKYYGNKLNAHLDITDDYPNSRNKVVKLSLKPYRFDVYLDNGVYKFVTVKNLDVIKKENYYEVNSKCYEEAKKLKKISNQAEFIASFYNNDLIKINGELYRVIGVNNDLLNRIEVNMIDITYREYLENMNDKRPPRIIKTIASKTQSIKKYSTDILGNLYEVKSKKHPQIIKKGKRPAATKKAGQAKKKKGSDAKSLTAWSRTLVTFKDVFVDFTREEWKLLDTAQQIVYRNVMLENYKNLVSLGYQLTKPDVILRLEKGEEP

SEQ ID NO: 22 - protein, 1483 aa, Artificial Sequence
  Synthetic Polypeptide
MDKKYSIGLAIGTNSVGWAVITDEYKVPSKKFKVLGNTDRHSIKKNLIGALLFDSGETAEATRLKRTARRRYTRRKNRICYLQEIFSNEMAKVDDSFFHRLEESFLVEEDKKHERHPIFGNIVDEVAYHEKYPTIYHLRKKLVDSTDKADLRLIYLALAHMIKFRGHFLIEGDLNPDNSDVDKLFIQLVQTYNQLFEENPINASGVDAKAILSARLSKSRRLENLIAQLPGEKKNGLFGNLIALSLGLTPNFKSNFDLAEDAKLQLSKDTYDDDLDNLLAQIGDQYADLFLAAKNLSDAILLSDILRVNTEITKAPLSASMIKRYDEHHQDLTLLKALVRQQLPEKYKEIFFDQSKNGYAGYIDGGASQEEFYKFIKPILEKMDGTEELLVKLNREDLLRKQRTFDNGSIPHQIHLGELHAILRRQEDFYPFLKDNREKIEKILTFRIPYYVGPLARGNSRFAWMTRKSEETITPWNFEEVVDKGASAQSFIERMTNFDKNLPNEKVLPKHSLLYEYFTVYNELTKVKYVTEGMRKPAFLSGEQKKAIVDLLFKTNRKVTVKQLKEDYFKKIECFDSVEISGVEDRFNASLGTYHDLLKIIKDKDFLDNEENEDILEDIVLTLTLFEDREMIEERLKTYAHLFDDKVMKQLKRRRYTGWGRLSRKLINGIRDKQSGKTILDFLKSDGFANRNFMQLIHDDSLTFKEDIQKAQVSGQGDSLHEHIANLAGSPAIKKGILQTVKVVDELVKVMGRHKPENIVIEMARENQTTQKGQKNSRERMKRIEEGIKELGSQILKEHPVENTQLQNEKLYLYYLQNGRDMYVDQELDINRLSDYDVDAIVPQSFLKDDSIDNKVLTRSDKNRGKSDNVPSEEVVKKMKNYWRQLLNAKLITQRKFDNLTKAERGGLSELDKAGFIKRQLVETRQITKHVAQILDSRMNTKYDENDKLIREVKVITLKSKLVSDFRKDFQFYKVREINNYHHAHDAYLNAVVGTALIKKYPKLESEFVYGDYKVYDVRKMIAKSEQEIGKATAKYFFYSNIMNFFKTEITLANGEIRKRPLIETNGETGEIVWDKGRDFATVRKVLSMPQVNIVKKTEVQTGGFSKESILPKRNSDKLIARKKDWDPKKYGGFDSPTVAYSVLVVAKVEKGKSKKLKSVKELLGITIMERSSFEKNPIDFLEAKGYKEVKKDLIIKLPKYSLFELENGRKRMLASAGELQKGNELALPSKYVNFLYLASHYEKLKGSPEDNEQKQLFVEQHKHYLDEIIEQISEFSKRVILADANLDKVLSAYNKHRDKPIREQAENIIHLFTLTNLGAPAAFKYFDTTIDRKRYTSTKEVLDATLIHQSITGLYETRIDLSQLGGDGTGGPKKKRKVYPYDVPDYAGYPYDVPDYAGSYPYDVPDYAGSMDAKSLTAWSRTLVTFKDVFVDFTREEWKLLDTAQQIVYRNVMLENYKNLVSLGYQLTKPDVILRLEKGEEP

SEQ ID NO: 23 - protein, 1069 aa, Artificial Sequence
  Synthetic Polypeptide
MAPKKKRKVGIHGVPAAKRNYILGLAIGITSVGYGIIDYETRDVIDAGVRLFKEANVENNEGRRSKRGARRLKRRRRHRIQRVKKLLFDYNLLTDHSELSGINPYEARVKGLSQKLSEEEFSAALLHLAKRRGVHNVNEVEEDTGNELSTKEQISRNSKALEEKYVAELQLERLKKDGEVRGSINRFKTSDYVKEAKQLLKVQKAYHQLDQSFIDTYIDLLETRRTYYEGPGEGSPFGWKDIKEWYEMLMGHCTYFPEELRSVKYAYNADLYNALNDLNNLVITRDENEKLEYYEKFQIIENVFKQKKKPTLKQIAKEILVNEEDIKGYRVTSTGKPEFTNLKVYHDIKDITARKEIIENAELLDQIAKILTIYQSSEDIQEELTNLNSELTQEEIEQISNLKGYTGTHNLSLKAINLILDELWHTNDNQIAIFNRLKLVPKKVDLSQQKEIPTTLVDDFILSPVVKRSFIQSIKVINAIIKKYGLPNDIIIELAREKNSKDAQKMINEMQKRNRQTNERIEEIIRTTGKENAKYLIEKIKLHDMQEGKCLYSLEAIPLEDLLNNPFNYEVDHIIPRSVSFDNSFNNKVLVKQEEASKKGNRTPFQYLSSSDSKISYETFKKHILNLAKGKGRISKTKKEYLLEERDINRFSVQKDFINRNLVDTRYATRGLMNLLRSYFRVNNLDVKVKSINGGFTSFLRRKWKFKKERNKGYKHHAEDALIIANADFIFKEWKKLDKAKKVMENQMFEEKQAESMPEIETEQEYKEIFITPHQIKHIKDFKDYKYSHRVDKKPNRELINDTLYSTRKDDKGNTLIVNNLNGLYDKDNDKLKKLINKSPEKLLMYHHDPQTYQKLKLIMEQYGDEKNPLYKYYEETGNYLTKYSKKDNGPVIKKIKYYGNKLNAHLDITDDYPNSRNKVVKLSLKPYRFDVYLDNGVYKFVTVKNLDVIKKENYYEVNSKCYEEAKKLKKISNQAEFIASFYNNDLIKINGELYRVIGVNNDLLNRIEVNMIDITYREYLENMNDKRPPRIIKTIASKTQSIKKYSTDILGNLYEVKSKKHPQIIKKG

SEQ ID NO: 24 - DNA, 16 bp, Artificial Sequence
  Synthetic Polynucleotide
atgcttcgtgatgacc

SEQ ID NO: 25 - DNA, 16 bp, Artificial Sequence
  Synthetic Polynucleotide
atcagccttaattcga

SEQ ID NO: 26 - DNA, 16 bp, Artificial Sequence
  Synthetic Polynucleotide
cagcgtcggaaggtgg

SEQ ID NO: 27 - DNA, 15 bp, Artificial Sequence
  Synthetic Polynucleotide
aacacgtctatacgc

SEQ ID NO: 28 - DNA, 23 bp, Artificial Sequence
  Synthetic Polynucleotide
gctctgctggaggagctttagga

SEQ ID NO: 29 - DNA, 20 bp, Artificial Sequence
  Synthetic Polynucleotide
gcaggtctgcwggtacctgg

SEQ ID NO: 30 - DNA, 19 bp, Artificial Sequence
  Synthetic Polynucleotide
tcgtggacagcatcacagt

SEQ ID NO: 31 - DNA, 19 bp, Artificial Sequence
  Synthetic Polynucleotide
cttcctagcatcagggcag

SEQ ID NO: 32 - DNA, 21 bp, Artificial Sequence
  Synthetic Polynucleotide
gtagcaggtgtaaccgtaacc

SEQ ID NO: 33 - DNA, 22 bp, Artificial Sequence
  Synthetic Polynucleotide
cagagataaatacagccccagg

SEQ ID NO: 34 - DNA, 20 bp, Artificial Sequence
  Synthetic Polynucleotide
acagaagcgcaatgttgaag

SEQ ID NO: 35 - DNA, 20 bp, Artificial Sequence
  Synthetic Polynucleotide
cacctttgcttgcagtttgt

SEQ ID NO: 36 - DNA, 22 bp, Artificial Sequence
  Synthetic Polynucleotide
tctacagagacgtaggctgtca

SEQ ID NO: 37 - DNA, 20 bp, Artificial Sequence
  Synthetic Polynucleotide
cttgagcacgagcttggtag

SEQ ID NO: 38 - DNA, 21 bp, Artificial Sequence
  Synthetic Polynucleotide
agtaagtgcgggtcataagct

SEQ ID NO: 39 - DNA, 22 bp, Artificial Sequence
  Synthetic Polynucleotide
cctcactaaaccatccaatcgg

SEQ ID NO: 40 - DNA, 20 bp, Artificial Sequence
  Synthetic Polynucleotide
tgcgacagtgtattcgcaac

SEQ ID NO: 41 - DNA, 20 bp, Artificial Sequence
  Synthetic Polynucleotide
ggctttggtcctcgtttctt

SEQ ID NO: 42 - DNA, 20 bp, Artificial Sequence
  Synthetic Polynucleotide
gctcattccagcaccaattc

SEQ ID NO: 43 - DNA, 20 bp, Artificial Sequence
  Synthetic Polynucleotide
ccattcatccacaccctcat

SEQ ID NO: 44 - DNA, 20 bp, Artificial Sequence
  Synthetic Polynucleotide
aaacactcaagccatccaca

SEQ ID NO: 45 - DNA, 21 bp, Artificial Sequence
  Synthetic Polynucleotide
gcttttctaattcccgctttt

SEQ ID NO: 46 - DNA, 20 bp, Artificial Sequence
  Synthetic Polynucleotide
caccgaaagccgtttgtgag

SEQ ID NO: 47 - DNA, 20 bp, Artificial Sequence
  Synthetic Polynucleotide
tctacccgtcacagcacaac

SEQ ID NO: 48 - DNA, 19 bp, Artificial Sequence
  Synthetic Polynucleotide
tctgctggaggagctttag

SEQ ID NO: 49 - DNA, 18 bp, Artificial Sequence
  Synthetic Polynucleotide
gaatggcagttctccgcg

SEQ ID NO: 50 - DNA, 20 bp, Artificial Sequence
  Synthetic Polynucleotide
cctatacccaccagcttctt

SEQ ID NO: 51 - DNA, 20 bp, Artificial Sequence
  Synthetic Polynucleotide
gatgtgattccccttctttc

SEQ ID NO: 52 - DNA, 20 bp, Artificial Sequence
  Synthetic Polynucleotide
atctggttgtggtagtgtgc

SEQ ID NO: 53 - DNA, 20 bp, Artificial Sequence
  Synthetic Polynucleotide
tgagggtgtctgaaagaatg

SEQ ID NO: 54 - DNA, 20 bp, Artificial Sequence
  Synthetic Polynucleotide
tgggaaatacctgctacgtg

SEQ ID NO: 55 - DNA, 20 bp, Artificial Sequence
  Synthetic Polynucleotide
gtgacgatgacacgtttgag